European Patent Application EP 4 248 961 A1, published September 27, 2023. Title: Antiviral composition against SARS-CoV-2 and HCoV-OC43 comprising rhein, meclofenamic acid, or combination thereof. Applicant: Seoul National University R&DB Foundation INSTITUTE FOR BASIC SCIENCE. The sequence listing filed with the application follows.

SEQUENCE LISTING (12 sequences)

SEQ ID NO: 1 - DNA, 20 bp, Artificial Sequence
  qPCR-nsp12-F: Forward primer sequence for qPCR against nsp12 in SARS-CoV-2-infected cells
cagagagctaggtgttgtac

SEQ ID NO: 2 - DNA, 20 bp, Artificial Sequence
  qPCR-nsp12-R: Reverse primer sequence for qPCR against nsp12 in SARS-CoV-2-infected cells
aagcacgtagtgcgtttatc

SEQ ID NO: 3 - DNA, 21 bp, Artificial Sequence
  qPCR-M-F: Forward primer sequence for qPCR against M in SARS-CoV-2-infected cells
cgtgccactccatggcactat

SEQ ID NO: 4 - DNA, 22 bp, Artificial Sequence
  qPCR-M-R: Reverse primer sequence for qPCR against M in SARS-CoV-2-infected cells
cgtcctagatggtgtccagcaa

SEQ ID NO: 5 - DNA, 20 bp, Artificial Sequence
  qPCR-N-F: Forward primer sequence for qPCR against N in SARS-CoV-2-infected cells
ggccagaagctggacttccc

SEQ ID NO: 6 - DNA, 20 bp, Artificial Sequence
  qPCR-N-R: Reverse primer sequence for qPCR against N in SARS-CoV-2-infected cells
aggattgcgggtgccaatgt

SEQ ID NO: 7 - DNA, 22 bp, Artificial Sequence
  qPCR-GAPDH-F: Forward primer sequence for qPCR against GAPDH in Calu-3 and HBEC cells
ctctctgctcctcctgttcgac

SEQ ID NO: 8 - DNA, 19 bp, Artificial Sequence
  qPCR-GAPDH-R: Reverse primer sequence for qPCR against GAPDH in Calu-3 and HBEC cells
tgagcgatgtggctcggct

SEQ ID NO: 9 - DNA, 19 bp, Artificial Sequence
  qPCR-GAPDH-F: Forward primer sequence for qPCR against GAPDH in Vero and HCT-8 cells
tgccaacgtgtcagtggtg

SEQ ID NO: 10 - DNA, 21 bp, Artificial Sequence
  qPCR-GAPDH-R: Reverse primer sequence for qPCR against GAPDH in Vero and HCT-8 cells
gcctgcttcaccaccttcttg

SEQ ID NO: 11 - DNA, 22 bp, Artificial Sequence
  qPCR-OC43-N-F: Forward primer sequence for qPCR against N in HCoV-OC43-infected cells
taagcaatccagtagtagagcg

SEQ ID NO: 12 - DNA, 20 bp, Artificial Sequence
  qPCR-OC43-N-R: Reverse primer sequence for qPCR against N in HCoV-OC43-infected cells
tctaaactggtcggactgat